European Patent Specification EP 3 365 005 B1, published April 9, 2025. Title: RECOMBINANT MOPEIA VIRUS AND VACCINE PLATFORM. Applicant: INSTITUT PASTEUR. The sequence listing filed with the application follows.

SEQUENCE LISTING (21 sequences)

SEQ ID NO: 1 - DNA, 6588 bp, Mopeia mammarenavirus
ggagatggggcagatagtcaccttctttcaagaggtgccacacatccttgaagaagtgatgaacattgtgctgatgaccctctcaatcttggccatcctaaagggcatctacaatgtgatgacctgtggaatcatcggtttgataacatttttgttcttgtgtgggagatcatgctcaagcatctataaggacaactatgagttcttctctctcgacctcgacatgtcttcactgaatgcaacgatgcctctctcctgctcaaagaacaactcccatcactacatccaagttgggaatgagacaggcctagagctgacattgacaaacactagcataattgatcataagttttgcaacctgtctgatgctcacaggaggaatctttatgacaaagcacttatgtcaatcttgacaacattccacctaagcattccagattttaaccaatatgaggcaatgtcatgtgattttaacggagggaagatctcaattcaatacaacctgtcccactcaaattatgtggatgccggcaaccactgtggcactattgcaaatggcattatggatgtttttagaagaatgtattggagcacctccctttcggttgcctctgacataagtgggactcaatgcatacagaccgattataagtatttgattattcagaacacatcatgggaggatcattgcatgttctcaagaccctcacccatgggatttttaagccttctgtcacagagaaccaggaatttctacatctcaagaagacttttgggtctttttacatggactttgagtgactcggaagggaacgacatgccaggtggttactgtctcacaaggtctatgctaatagggcttgatctgaaatgctttgggaacactgccattgcgaagtgtaatcaggcacatgatgaagaattctgtgacatgctccgcctttttgattttaataaacaagcaattagcaaactgaggtctgaagttcagcagagcataaatttgataaataaagctgtcaacgccctcatcaatgatcaactggtcatgaggaaccatttgagagatctaatgggtattccttattgcaactactctaagttttggtacttgaatgatactaggacagggagaacatccctcccaaagtgttggcttgtgaccaatgggtcatacctaaatgaaacccagttctcaacagaaattgagcaagaagccaataacatgttcactgacatgttgaggaaggagtatgagaaaaggcagagcacaacacctctggggttagtagatctttttgttttctccactagcttttatttgatctccgtgttcctccacctaatcaaaattccaacacatagacacataaaaggcaagccttgcccgaaaccacacagactcaatcacatggcaatctgttcctgtggcttctataagcaaccaggtctccccacacaatggaaaaggtgaagaacaggggcacccccgagacccaccgccttcggcggtgggtctcgggggcctggagtgactgttccttgatggcctccacgacccaccgccagaggcggtgggtcgtggaggtgtcccttcttacaggacaactctgggaggacctgttctaaacaccaggtctctactcaagactggtctgggggttggaatttgtggactccctatgactgctgcttcaaacatgagacaatccagcaatgcacagtgtggtgtcacttcttctttgccacctctcttcttcttttgcgttacaatccccgtatgcattctacaaaggtgtttgtattcatcccagatcttatcctcaaattttcttgcatcgtctttctgcatggacacatcaatcagttttatgtccctcctgttctgggagtcaagaagctttctgatgtcatcagcaccttgacacgacaagaccatgttctttggcaggctctcaattacagcacttgtcaaccccggctgaactgagaataggtcttggatgtcaatgccatgagagtgtttggagtcttgtttgaattgtttaatgtctgttggttccctgtaaaaatgaatatactgaccattattaggttgatagatagctatctccacggggtcttcaggtctcccttctatgtcaatccatgtcttagcatttggatccaattgcaacatgctgtctttgagttccattgtctgagagtaggtcaaaccagcaggcatgccttgggcctgagcgagtctgttggagttacctttgtcaggctttgcattctgttgcacatcaccactcagatcaacagttgtgttatcccaagccctgccgacgatcgatgttcttgatgctatgtaaggccaaccctctccagaaagacatagtttgtagaggagattttcataagggttcctttcccctggcgtgtcagagacaaacattcccaaagaacgcttgactttcaaggcagccttcaaaattccttccaaattggattttgttactttgatggtctccagcatgtttccgccgtctattagacaagcaccagctttcaccgcagctgacaggctaaaattgtaccctgatatgtttatggcacttttcttgggctcaatgatccccaagattgggtgggtctgagagagtttgtctaagtcagacatgtttggatactttgcagtgtacacaagccccaagtctgacaacgattggatcacatcattcagatctgcctgcccttgtttgcacatgcaagcaatcgtcaggcttggcattgtcccaaactgattgtttaaaagctctgggtttcgaacatcccacactctaacaatgccatctccgagagtgtttcctgcccggaacccgccacccattccgaccatctgtaacaaaaccctcctctgttctagctgctgagctgttaggttgcccatatagactccagcagcaagaggcctctcacctctgatgacttttgctttgagtctgtccaggtcggcagcaaggacgaggaggtcatcagaggttagtgtccccactctcaaaacattcttctgttggactgactttaactcaactagattgttcactgcctggtttaggtccctcaatcttttcaggtcagagtcatccctcttctcctttctcatcaacctttgaacattggcaacttcagagaagtccagcccatgaagaagtgcttgagcatccttgatgacttggatctttatgttggagcagtaccctgagagttctctcctcaggctctgtgtccacaagaaggacttcacctcctttgaattggacattgttggaggcttttcggtgcagagtctcaatcttggccatcctaaagggcatctacaatgtgatgacctgtggaatcatcggtttgataacatttttgttcttgtgtgggagatcatgctcaagcatctataaggacaactatgagttcttctctctcgacctcgacatgtcttcactgaatgcaacgatgcctctctcctgctcaaagaacaactcccatcactacatccaagttgggaatgagacaggcctagagctgacattgacaaacactagcataattgatcataagttttgcaacctgtctgatgctcacaggaggaatctttatgacaaagcacttatgtcaatcttgacaacattccacctaagcattccagattttaaccaatatgaggcaatgtcatgtgattttaacggagggaagatctcaattcaatacaacctgtcccactcaaattatgtggatgccggcaaccactgtggcactattgcaaatggcattatggatgtttttagaagaatgtattggagcacctccctttcggttgcctctgacataagtgggactcaatgcatacagaccgattataagtatttgattattcagaacacatcatgggaggatcattgcatgttctcaagaccctcacccatgggatttttaagccttctgtcacagagaaccaggaatttctacatctcaagaagacttttgggtctttttacatggactttgagtgactcggaagggaacgacatgccaggtggttactgtctcacaaggtctatgctaatagggcttgatctgaaatgctttgggaacactgccattgcgaagtgtaatcaggcacatgatgaagaattctgtgacatgctccgcctttttgattttaataaacaagcaattagcaaactgaggtctgaagttcagcagagcataaatttgataaataaagctgtcaacgccctcatcaatgatcaactggtcatgaggaaccatttgagagatctaatgggtattccttattgcaactactctaagttttggtacttgaatgatactaggacagggagaacatccctcccaaagtgttggcttgtgaccaatgggtcatacctaaatgaaacccagttctcaacagaaattgagcaagaagccaataacatgttcactgacatgttgaggaaggagtatgagaaaaggcagagcacaacacctctggggttagtagatctttttgttttctccactagcttttatttgatctccgtgttcctccacctaatcaaaattccaacacatagacacataaaaggcaagccttgcccgaaaccacacagactcaatcacatggcaatctgttcctgtggcttctataagcaaccaggtctccccacacaatggaaaaggtgaagaacaggggcacccccgagacccaccgccttcggcggtgggtctcgggggcctggagtgactgttccttgatggcctccacgacccaccgccagaggcggtgggtcgtggaggtgtcccttcttacaggacaactctgggaggacctgttctaaacaccaggtctctactcaagactggtctgggggttggaatttgtggactccctatgactgctgcttcaaacatgagacaatccagcaatgcacagtgtggtgtcacttcttctttgccacctctcttcttcttttgcgttacaatccccgtatgcattctacaaaggtgtttgtattcatcccagatcttatcctcaaattttcttgcatcgtctttctgcatggacacatcaatcagttttatgtccctcctgttctgggagtcaagaagctttctgatgtcatcagcaccttgacacgacaagaccatgttctttggcaggctctcaattacagcacttgtcaaccccggctgaactgagaataggtcttggatgtcaatgccatgagagtgtttggagtcttgtttgaattgtttaatgtctgttggttccctgtaaaaatgaatatactgaccattattaggttgatagatagctatctccacggggtcttcaggtctcccttctatgtcaatccatgtcttagcatttggatccaattgcaacatgctgtctttgagttccattgtctgagagtaggtcaaaccagcaggcatgccttgggcctgagcgagtctgttggagttacctttgtcaggctttgcattctgttgcacatcaccactcagatcaacagttgtgttatcccaagccctgccgacgatcgatgttcttgatgctatgtaaggccaaccctctccagaaagacatagtttgtagaggagattttcataagggttcctttcccctggcgtgtcagagacaaacattcccaaagaacgcttgactttcaaggcagccttcaaaattccttccaaattggattttgttactttgatggtctccagcatgtttccgccgtctattagacaagcaccagctttcaccgcagctgacaggctaaaattgtaccctgatatgtttatggcacttttcttgggctcaatgatccccaagattgggtgggtctgagagagtttgtctaagtcagacatgtttggatactttgcagtgtacacaagccccaagtctgacaacgattggatcacatcattcagatctgcctgcccttgtttgcacatgcaagcaatcgtcaggcttggcattgtcccaaactgattgtttaaaagctctgggtttcgaacatcccacactctaacaatgccatctccgagagtgtttcctgcccggaacccgccacccattccgaccatctgtaacaaaaccctcctctgttctagctgctgagctgttaggttgcccatatagactccagcagcaagaggcctctcacctctgatgacttttgctttgagtctgtccaggtcggcagcaaggacgaggaggtcatcagaggttagtgtccccactctcaaaacattcttctgttggactgactttaactcaactagattgttcactgcctggtttaggtccctcaatcttttcaggtcagagtcatccctcttctcctttctcatcaacctttgaacattggcaacttcagagaagtccagcccatgaagaagtgcttgagcatccttgatgacttggatctttatgttggagcagtaccctgagagttctctcctcaggctctgtgtccacaagaaggacttcacctcctttgaattggacattgttggaggcttttcggtgcagag

SEQ ID NO: 2 - DNA, 14462 bp, Mopeia mammarenavirus
cgcaccggggatcctaggcaattttgtggatctttgctgatacttcattctgcactcaaagccgcatccggcaagagtcatggggaaaacgcagtccaagggacagcccagcacaaatctcctcaaggagacagaaccaaggcatccagtaataccagatgccaggggaactggccctgaattctgcaagagctgctggttcgaaaggagggggttagtcaggtgcaacgatcactacctatgtttgaactgtcttacacttttacacacagtgtcagataggtgccccatctgcaaacacaaactacccttcagactagagctccagacccagccgacagcaccaccagaaatcccaccatcccaaaatcccccaccctacagcccctgaggcagaactccgccccgaagcccctcccaaacacccctcccctcccccccggggggaccccccgccggggctccccccggggggagatgcgcgagctgttctcggagcacctactcaatgtcgaggggaggccccacctcttcaaagaggggcctgcacagcctccctcttaatctaaacttcccctctgaagactggatcatcagtgaagcctgcgatctactgtagcagagactatagcctttaaaatctgcccagaagtcaattccggagaacactctagtaaggaagttttcgtagccttcaggcatgcatcgtcccacaacccctataatatcaagttgtagccagtgtagtccttggtccattctggatctcagcatcttgctcaaagatctctccaagatttcggaatgatcctccattagctcaccaataaaaacattaagatcctggtcatggatgttggggttgaagggcaggagtttcctggtcccttcaataaggtatcctgagtcaacaactaaggggatttcaacatgctcaggccctatatgcgtgaaatcatgttcctccaggtccaggatctcctcattcaataagacggacaagggtatcacatcaggaatgggggaactatccctcaagtagtcacaaatattttcagtggacagcaaccaaattgatgtggtttcccttttaaaccatgtagatgtctgtgcaactctccagcaatctttaattgcggatctttgaacactaccactgtaagttacatcaagggaatgaggcttgaataatccaccttccaacaccacccctttgaaaaggaggtggagactaaatttctctttcaatgattcaccctgacttctcacctgaaaatttactgtgacagaaatttgaacgctcccaacactgaggtcggcaaaagcttcaagcagctcacttaccgactcaaagacgtgctgctcggttaatcctgatgctatgagctgtcctaagtttagaattgctggtgcacattcaaaatccagccaagcataacctgagtaaagatcatgcctgtacatgggtctttcaacacccttataaataaccttttctataaaagaagaaaaggggccgaggttgtcaagcccttccgactcaggaattgaagatctatgtggaaaccaagtaaaagaacctaaagtcctgcttgttgcaacgaatggtctgatgaaggactcaaagtagatttgtctcaggaaattttgtaccacatcataagtggtcaccaccctttcatccgtgattgggagatgagacctctcatgtgctattgctaaatctgaagacagaaccacataatgctcttctctcttccacttgacaacatgagaaattaatgacattgcctcacaattcacatctagaaccacacaaagatcaagaaacttaatccttggtgtccacctcattttcgttgatgctaggtcactcatgaagggcaagaggtgtctctcaaatagagatgggtaaagtcttctgaatgagtgaataatatggttaaaccccaccttgtcttccaagagttttgtggtagtgggcttcattgggaaatagtcacatggcttgaagggaattgaggatgttttctccttcactttgggttcacccaacacccaggaacccagctcaagtgatgtagataaggctatgcagaagtaatcccaaaggacaggtctcaagaaacctaacgcttcctcagctgcctttgtgtgctccttacccaagatccaaagatcgacgcccttaactttcaagctggaaacagaatccaatgctgacagtcttgaaactaatgattttatataggcggtggacctatctgagaatcgaacacatttgctacctagtgtcttgcaaagacctatgaaacctgatgctatcccactctgaaaggcacttttgttgacggcttcacagagcaacttttgtgcccctcttgtgaaattagaggataacttgctttgcaatgttttcaccaaggtaggcagtttttcttccccgagttcaacagcacctgtgtaaatgaccttctgtctcatgaccatctttaaagggtgatgagttgtcaaattaagccaacacaccgataaatcctcttctgagagggtgtcatcaccaacaaggctggtaagtttcttgaaggaatctgcggggtctcctgacaagtagatggctgtgaattcttcatgaagctctcctaatttcagcttattaaaaactgtccttaggaccttcctaactttctgagtgctttctggtaggattgcctcaatgttcctcataatcctatagcccctattgccatcaacccaatctttaacatcagaatccaaaaacaacaagaaaggatcaatgggatattgtgcatatctaagtagattcagtgttctctcctgaatagcgttacatagtgtgacaggcacaccattggccactgactgatcaatgatagtgtcaatagtttcagctaattgatgtggctccttacacttaacgttgtggagggcggcagccacgaatttcgttaacaatggaacttcatcaccccagacataaaaccttgatttgaactcagcaacaaatgaaccaataacactctttggactgatgaatttattcaattgatcacttaggaaatagtgaaattctagaatggcttggaattcctcaggctcatttgagagtaaatctgaaagatccttgccaaatagtgatatttgatcatcactagaggtatatgaatcaacttcatcttcaaatagacacttaatgcaataatttatgaatctctcactcactagaccgtagaagtcagaagcattgtgcaagatcccttgccccatgtcaattattgagctgagatgtgatggtatcctgttttgtttaaagtattcaaagaagaaagcttctgttgacgtttggtggagtgattttttcaaacctaacctagacttaagataagatctcatcattgcattcacaacattgaaaggtacctcaattaacttgtgaatgtgccacgacagcaaagtggacacgtaatccttactttttatgtcctctatatcatctcctgtctcccatcgcaaattttgaagaaacaccaggaaaagaaaaggggacatcataggcccccacttgctgtgatcgaggctataagagacctgacctagtgaaacattcaatttcatggctagaatggcattgtggaattccttttcattattaagacagctccctctatattgcttagttagtgcctcaaaataatcctcaattaggcgtgtgaacatttttgtcctcaggtcacctatataaagttccctgttccctccaacttgttctttgtaagataaggaaaacttgagccttccagtatcaggacccaaggatgtgtatgactgtggggattcttgactgtaaaaacataggttctttagaactgcagttgtacaatttgtcaatgacagtgctttacctaatgcctcagaattgctctctctttcactgatcctaacatcattcatcagcctttctctatcaatcttgaagtttaagcatttgtttttgtaatggctgtattttccagccaatttccctgcattcatctgaagaagtagtgacttgaagcactgaaaaaactgctggtcattgaatgttctggtggagacagcttgggtgatgcatgttattgggcaagagtccaaggaatccaaatagaaatactttgaccttaactccaaatccttaaaaaagcctttgcagatcatctcataagcatctccaggtagtagtgactcatcaaaatcttccaccatgtggtgtgctatctctgcctggatcagtctgtagtaaacacagcccacatcttcagtacctaaaaccttcctcaagtctgtcaaggacttctcctctgacccatttcccacagggaacttcctgtcatatctatacttctcaaggacgacatcaacagatttcttcacatcctctagacagtcaagtgcacaactatccaagaataactcatctaattcgtcaggagccccttgtgaattgggatttgaggaacctgacttcttccccacaacaaggtcactaatggccttttgcaccttataatcataatcctccttactcaagaggtatttagttttcctctggaatacctctgatagctggcaaacagaagcagccactagtttatcatgatcgtaattaagtatcctctctccgtcagtatacttattcacaaccacacttttgttgcttgcaaggtcaagagctgttgcacacccagcagtaactaatggatctttaaacccacttaggtcatctcctttcttgaaaagagagccattgttaaaagaagacgtcatcattgagaagaattttcttgacacaccaggaactttataagatattctgttgttactcatactggtttctttggataaaaatttgtttgctgattcaagcagcagcatcctttcatcttcatccccctcttcagatgggttgatgttaatactgtcaaactccaacttgggctccaaatacttctcaaagcacttaatctgatctgtcaacctatctggagtttccttagttataaaatgacacatgtatgataggtttaacacaaacttaaatctattagtcaacatagtgctcaccccttcacccaggatgatgttgagaatgctcctcaccacactatacaagaggtgctccggctctgttatgagatcctccctcaacttttccattaactgcttatggtggaagtctgaaacaaaggccattatgaagtatcgcagaccttgcaagaacttctgtgctcttttgctagggttcacaagtatgaggatcatggtgattttgagcaataattttaaagttttttgttgatctctgagttctatacattcagacaaccaactcatcatggtgttgatagtctcatagataacacagtgtgagaaaattgcaggaaaaaacctttttggatctgcatagaatgaacaaatctcccccttctcaggattgttaatggcataacattttgagcactctcctgttttctgataaattaagttgaaattcccgcttcccatgataaagctttgattaaaagcttccttacaacgtacacgtttgtaccttgcagcaccatactcattttgcctcactttggctactgatgatgtcttcattgaattcaccaatgccaaagagatgctagatagtcttctcaggtcttctatggaatcagcttccaactcaataagagggtaggggaattgattcccctcttctttctcatagctcattgttggctgaatccctcttttctccattaacataagcctctcgtaactgtcctcctccagtatatcttcctctttaacataatctctaaagcacaaactggcagaggataatgcctctttggcctttgtgaggagtttgtttatgatgtcaaagaatataagctcagatctctgacacagagttcctacacctcccttcttcttcattgcactcaccattctcctttcaatccactttttaaggtccttttgtgtttcttgtagtgacaccaatctgtcgttcacacttaagaatgaggagccaagccattctgatcctaacagctcgccgtgacatttaagatcctttaagtgggccaaaaggatgattgcgtcaaaagtcagcattagttttcttctggtgttcaataactttagtgattttattttattcaacagtgacttccatccaggcacagagctttggaagtgattctgcaagcagctgtctcgatcaactccctcttgcctataacggtcgtagtcaccatagagcgctgttaccataggcgaggattttacaaacctctcttttagaggatcaatctctgagggtgtgtccccctctctgtcaatataaaggttgttgaaatctctcaagagctgtcgcctatctgtcctgacaaattgtctttctatctcaccctctttaagcttattcctaaaagcatgaaattctgatacaatctcttttttcacatcaagaatggacattttgttattgatgcctctgtggcagagctccaacaccctctcataatgatcagatcgagaatctgtcaaaacattgaggctctcaatgcccgatgttctcactcctgcttttgttaaagattcacaaagccttgagtactcagattcttcaaacatttttgatgactgctgcgagaattcaagtaagctaaataggatatgcctaaacctctcattggcccattctggaaacaaatcagtgtagaaattggttctgccgtctatcaagggcaacagaatgatgtcaacagatgataagtcaggctttaaagactctagcttaatggtatcttctttatacttttgctcaaagtttattggtgaagtcctgacaaagcattccagtaatattaatgtgttcccactgaatttgaatccatctggcaccacaaatggtagaccagggcacagaacaccttgtctctgcagaaggatttcaacagaaaggtcttctgagttgtgctcacaaccattggctttgcaactgtctatctcaatacagagtgacaacaacttaaggccctcaattaatagcattctcggctctgtctgaactaggaaggctagcttctgttttgaaagcctctcatcctctaagaggtacctgctcacaagatctttgctctcggacagcaactcctccatcaccacacacttgttcctcagaagagagagtcacaatgcctaggatcctcggtgcgtggggaaaacgcagtccaagggacagcccagcacaaatctcctcaaggagacagaaccaaggcatccagtaataccagatgccaggggaactggccctgaattctgcaagagctgctggttcgaaaggagggggttagtcaggtgcaacgatcactacctatgtttgaactgtcttacacttttacacacagtgtcagataggtgccccatctgcaaacacaaactacccttcagactagagctccagacccagccgacagcaccaccagaaatcccaccatcccaaaatcccccaccctacagcccctgaggcagaactccgccccgaagcccctcccaaacacccctcccctcccccccggggggaccccccgccggggctccccccggggggagatgcgcgagctgttctcggagcacctactcaatgtcgaggggaggccccacctcttcaaagaggggcctgcacagcctccctcttaatctaaacttcccctctgaagactggatcatcagtgaagcctgcgatctactgtagcagagactatagcctttaaaatctgcccagaagtcaattccggagaacactctagtaaggaagttttcgtagccttcaggcatgcatcgtcccacaacccctataatatcaagttgtagccagtgtagtccttggtccattctggatctcagcatcttgctcaaagatctctccaagatttcggaatgatcctccattagctcaccaataaaaacattaagatcctggtcatggatgttggggttgaagggcaggagtttcctggtcccttcaataaggtatcctgagtcaacaactaaggggatttcaacatgctcaggccctatatgcgtgaaatcatgttcctccaggtccaggatctcctcattcaataagacggacaagggtatcacatcaggaatgggggaactatccctcaagtagtcacaaatattttcagtggacagcaaccaaattgatgtggtttcccttttaaaccatgtagatgtctgtgcaactctccagcaatctttaattgcggatctttgaacactaccactgtaagttacatcaagggaatgaggcttgaataatccaccttccaacaccacccctttgaaaaggaggtggagactaaatttctctttcaatgattcaccctgacttctcacctgaaaatttactgtgacagaaatttgaacgctcccaacactgaggtcggcaaaagcttcaagcagctcacttaccgactcaaagacgtgctgctcggttaatcctgatgctatgagctgtcctaagtttagaattgctggtgcacattcaaaatccagccaagcataacctgagtaaagatcatgcctgtacatgggtctttcaacacccttataaataaccttttctataaaagaagaaaaggggccgaggttgtcaagcccttccgactcaggaattgaagatctatgtggaaaccaagtaaaagaacctaaagtcctgcttgttgcaacgaatggtctgatgaaggactcaaagtagatttgtctcaggaaattttgtaccacatcataagtggtcaccaccctttcatccgtgattgggagatgagacctctcatgtgctattgctaaatctgaagacagaaccacataatgctcttctctcttccacttgacaacatgagaaattaatgacattgcctcacaattcacatctagaaccacacaaagatcaagaaacttaatccttggtgtccacctcattttcgttgatgctaggtcactcatgaagggcaagaggtgtctctcaaatagagatgggtaaagtcttctgaatgagtgaataatatggttaaaccccaccttgtcttccaagagttttgtggtagtgggcttcattgggaaatagtcacatggcttgaagggaattgaggatgttttctccttcactttgggttcacccaacacccaggaacccagctcaagtgatgtagataaggctatgcagaagtaatcccaaaggacaggtctcaagaaacctaacgcttcctcagctgcctttgtgtgctccttacccaagatccaaagatcgacgcccttaactttcaagctggaaacagaatccaatgctgacagtcttgaaactaatgattttatataggcggtggacctatctgagaatcgaacacatttgctacctagtgtcttgcaaagacctatgaaacctgatgctatcccactctgaaaggcacttttgttgacggcttcacagagcaacttttgtgcccctcttgtgaaattagaggataacttgctttgcaatgttttcaccaaggtaggcagtttttcttccccgagttcaacagcacctgtgtaaatgaccttctgtctcatgaccatctttaaagggtgatgagttgtcaaattaagccaacacaccgataaatcctcttctgagagggtgtcatcaccaacaaggctggtaagtttcttgaaggaatctgcggggtctcctgacaagtagatggctgtgaattcttcatgaagctctcctaatttcagcttattaaaaactgtccttaggaccttcctaactttctgagtgctttctggtaggattgcctcaatgttcctcataatcctatagcccctattgccatcaacccaatctttaacatcagaatccaaaaacaacaagaaaggatcaatgggatattgtgcatatctaagtagattcagtgttctctcctgaatagcgttacatagtgtgacaggcacaccattggccactgactgatcaatgatagtgtcaatagtttcagctaattgatgtggctccttacacttaacgttgtggagggcggcagccacgaatttcgttaacaatggaacttcatcaccccagacataaaaccttgatttgaactcagcaacaaatgaaccaataacactctttggactgatgaatttattcaattgatcacttaggaaatagtgaaattctagaatggcttggaattcctcaggctcatttgagagtaaatctgaaagatccttgccaaatagtgatatttgatcatcactagaggtatatgaatcaacttcatcttcaaatagacacttaatgcaataatttatgaatctctcactcactagaccgtagaagtcagaagcattgtgcaagatcccttgccccatgtcaattattgagctgagatgtgatggtatcctgttttgtttaaagtattcaaagaagaaagcttctgttgacgtttggtggagtgattttttcaaacctaacctagacttaagataagatctcatcattgcattcacaacattgaaaggtacctcaattaacttgtgaatgtgccacgacagcaaagtggacacgtaatccttactttttatgtcctctatatcatctcctgtctcccatcgcaaattttgaagaaacaccaggaaaagaaaaggggacatcataggcccccacttgctgtgatcgaggctataagagacctgacctagtgaaacattcaatttcatggctagaatggcattgtggaattccttttcattattaagacagctccctctatattgcttagttagtgcctcaaaataatcctcaattaggcgtgtgaacatttttgtcctcaggtcacctatataaagttccctgttccctccaacttgttctttgtaagataaggaaaacttgagccttccagtatcaggacccaaggatgtgtatgactgtggggattcttgactgtaaaaacataggttctttagaactgcagttgtacaatttgtcaatgacagtgctttacctaatgcctcagaattgctctctctttcactgatcctaacatcattcatcagcctttctctatcaatcttgaagtttaagcatttgtttttgtaatggctgtattttccagccaatttccctgcattcatctgaagaagtagtgacttgaagcactgaaaaaactgctggtcattgaatgttctggtggagacagcttgggtgatgcatgttattgggcaagagtccaaggaatccaaatagaaatactttgaccttaactccaaatccttaaaaaagcctttgcagatcatctcataagcatctccaggtagtagtgactcatcaaaatcttccaccatgtggtgtgctatctctgcctggatcagtctgtagtaaacacagcccacatcttcagtacctaaaaccttcctcaagtctgtcaaggacttctcctctgacccatttcccacagggaacttcctgtcatatctatacttctcaaggacgacatcaacagatttcttcacatcctctagacagtcaagtgcacaactatccaagaataactcatctaattcgtcaggagccccttgtgaattgggatttgaggaacctgacttcttccccacaacaaggtcactaatggccttttgcaccttataatcataatcctccttactcaagaggtatttagttttcctctggaatacctctgatagctggcaaacagaagcagccactagtttatcatgatcgtaattaagtatcctctctccgtcagtatacttattcacaaccacacttttgttgcttgcaaggtcaagagctgttgcacacccagcagtaactaatggatctttaaacccacttaggtcatctcctttcttgaaaagagagccattgttaaaagaagacgtcatcattgagaagaattttcttgacacaccaggaactttataagatattctgttgttactcatactggtttctttggataaaaatttgtttgctgattcaagcagcagcatcctttcatcttcatccccctcttcagatgggttgatgttaatactgtcaaactccaacttgggctccaaatacttctcaaagcacttaatctgatctgtcaacctatctggagtttccttagttataaaatgacacatgtatgataggtttaacacaaacttaaatctattagtcaacatagtgctcaccccttcacccaggatgatgttgagaatgctcctcaccacactatacaagaggtgctccggctctgttatgagatcctccctcaacttttccattaactgcttatggtggaagtctgaaacaaaggccattatgaagtatcgcagaccttgcaagaacttctgtgctcttttgctagggttcacaagtatgaggatcatggtgattttgagcaataattttaaagttttttgttgatctctgagttctatacattcagacaaccaactcatcatggtgttgatagtctcatagataacacagtgtgagaaaattgcaggaaaaaacctttttggatctgcatagaatgaacaaatctcccccttctcaggattgttaatggcataacattttgagcactctcctgttttctgataaattaagttgaaattcccgcttcccatgataaagctttgattaaaagcttccttacaacgtacacgtttgtaccttgcagcaccatactcattttgcctcactttggctactgatgatgtcttcattgaattcaccaatgccaaagagatgctagatagtcttctcaggtcttctatggaatcagcttccaactcaataagagggtaggggaattgattcccctcttctttctcatagctcattgttggctgaatccctcttttctccattaacataagcctctcgtaactgtcctcctccagtatatcttcctctttaacataatctctaaagcacaaactggcagaggataatgcctctttggcctttgtgaggagtttgtttatgatgtcaaagaatataagctcagatctctgacacagagttcctacacctcccttcttcttcattgcactcaccattctcctttcaatccactttttaaggtccttttgtgtttcttgtagtgacaccaatctgtcgttcacacttaagaatgaggagccaagccattctgatcctaacagctcgccgtgacatttaagatcctttaagtgggccaaaaggatgattgcgtcaaaagtcagcattagttttcttctggtgttcaataactttagtgattttattttattcaacagtgacttccatccaggcacagagctttggaagtgattctgcaagcagctgtctcgatcaactccctcttgcctataacggtcgtagtcaccatagagcgctgttaccataggcgaggattttacaaacctctcttttagaggatcaatctctgagggtgtgtccccctctctgtcaatataaaggttgttgaaatctctcaagagctgtcgcctatctgtcctgacaaattgtctttctatctcaccctctttaagcttattcctaaaagcatgaaattctgatacaatctcttttttcacatcaagaatggacattttgttattgatgcctctgtggcagagctccaacaccctctcataatgatcagatcgagaatctgtcaaaacattgaggctctcaatgcccgatgttctcactcctgcttttgttaaagattcacaaagccttgagtactcagattcttcaaacatttttgatgactgctgcgagaattcaagtaagctaaataggatatgcctaaacctctcattggcccattctggaaacaaatcagtgtagaaattggttctgccgtctatcaagggcaacagaatgatgtcaacagatgataagtcaggctttaaagactctagcttaatggtatcttctttatacttttgctcaaagtttattggtgaagtcctgacaaagcattccagtaatattaatgtgttcccactgaatttgaatccatctggcaccacaaatggtagaccagggcacagaacaccttgtctctgcagaaggatttcaacagaaaggtcttctgagttgtgctcacaaccattggctttgcaactgtctatctcaatacagagtgacaacaacttaaggccctcaattaatagcattctcggctctgtctgaactaggaaggctagcttctgttttgaaagcctctcatcctctaagaggtacctgctcacaagatctttgctctcggacagcaactcctccatcaccacacacttgttcctcagaagagagagtcacaatgcctaggatcctcggtgcg

SEQ ID NO: 3 - protein, 489 aa, Mopeia mammarenavirus
MGQIVTFFQEVPHILEEVMNIVLMTLSILAILKGIYNVMTCGIIGLITFLFLCGRSCSSIYKDNYEFFSLDLDMSSLNATMPLSCSKNNSHHYIQVGNETGLELTLTNTSIIDHKFCNLSDAHRRNLYDKALMSILTTFHLSIPDFNQYEAMSCDFNGGKISIQYNLSHSNYVDAGNHCGTIANGIMDVFRRMYWSTSLSVASDISGTQCIQTDYKYLIIQNTSWEDHCMFSRPSPMGFLSLLSQRTRNFYISRRLLGLFTWTLSDSEGNDMPGGYCLTRSMLIGLDLKCFGNTAIAKCNQAHDEEFCDMLRLFDFNKQAISKLRSEVQQSINLINKAVNALINDQLVMRNHLRDLMGIPYCNYSKFWYLNDTRTGRTSLPKCWLVTNGSYLNETQFSTEIEQEANNMFTDMLRKEYEKRQSTTPLGLVDLFVFSTSFYLISVFLHLIKIPTHRHIKGKPCPKPHRLNHMAICSCGFYKQPGLPTQWKR

SEQ ID NO: 4 - protein, 570 aa, Mopeia mammarenavirus
MSNSKEVKSFLWTQSLRRELSGYCSNIKIQVIKDAQALLHGLDFSEVANVQRLMRKEKRDDSDLKRLRDLNQAVNNLVELKSVQQKNVLRVGTLTSDDLLVLAADLDRLKAKVIRGERPLAAGVYMGNLTAQQLEQRRVLLQMVGMGGGFRAGNTLGDGIVRVWDVRNPELLNNQFGTMPSLTIACMCKQGQADLNDVIQSLSDLGLVYTAKYPNMSDLDKLSQTHPILGIIEPKKSAINISGYNFSLSAAVKAGACLIDGGNMLETIKVTKSNLEGILKAALKVKRSLGMFVSDTPGERNPYENLLYKLCLSGEGWPYIASRTSIVGRAWDNTTVDLSGDVQQNAKPDKGNSNRLAQAQGMPAGLTYSQTMELKDSMLQLDPNAKTWIDIEGRPEDPVEIAIYQPNNGQYIHFYREPTDIKQFKQDSKHSHGIDIQDLFSVQPGLTSAVIESLPKNMVLSCQGADDIRKLLDSQNRRDIKLIDVSMQKDDARKFEDKIWDEYKHLCRMHTGIVTQKKKRGGKEEVTPHCALLDCLMFEAAVIGSPQIPTPRPVLSRDLVFRTGPPRVVL

SEQ ID NO: 5 - protein, 103 aa, Mopeia mammarenavirus
MGKTQSKGQPSTNLLKETEPRHPVIPDARGTGPEFCKSCWFERRGLVRCNDHYLCLNCLTLLHTVSDRCPICKHKLPFRLELQTQPTAPPEIPPSQNPPPYSP

SEQ ID NO: 6 - protein, 2237 aa, Mopeia mammarenavirus
MEELLSESKDLVSRYLLEDERLSKQKLAFLVQTEPRMLLIEGLKLLSLCIEIDSCKANGCEHNSEDLSVEILLQRQGVLCPGLPFVVPDGFKFSGNTLILLECFVRTSPINFEQKYKEDTIKLESLKPDLSSVDIILLPLIDGRTNFYTDLFPEWANERFRHILFSLLEFSQQSSKMFEESEYSRLCESLTKAGVRTSGIESLNVLTDSRSDHYERVLELCHRGINNKMSILDVKKEIVSEFHAFRNKLKEGEIERQFVRTDRRQLLRDFNNLYIDREGDTPSEIDPLKERFVKSSPMVTALYGDYDRYRQEGVDRDSCLQNHFQSSVPGWKSLLNKIKSLKLLNTRRKLMLTFDAIILLAHLKDLKCHGELLGSEWLGSSFLSVNDRLVSLQETQKDLKKWIERRMVSAMKKKGGVGTLCQRSELIFFDIINKLLTKAKEALSSASLCFRDYVKEEDILEEDSYERLMLMEKRGIQPTMSYEKEEGNQFPYPLIELEADSIEDLRRLSSISLALVNSMKTSSVAKVRQNEYGAARYKRVRCKEAFNQSFIMGSGNFNLIYQKTGECSKCYAINNPEKGEICSFYADPKRFFPAIFSHCVIYETINTMMSWLSECIELRDQQKTLKLLLKITMILILVNPSKRAQKFLQGLRYFIMAFVSDFHHKQLMEKLREDLITEPEHLLYSVVRSILNIILGEGVSTMLTNRFKFVLNLSYMCHFITKETPDRLTDQIKCFEKYLEPKLEFDSININPSEEGDEDERMLLLESANKFLSKETSMSNNRISYKVPGVSRKFFSMMTSSFNNGSLFKKGDDLSGFKDPLVTAGCATALDLASNKSVVVNKYTDGERILNYDHDKLVAASVCQLSEVFQRKTKYLLSKEDYDYKVQKAISDLVVGKKSGSSNPNSQGAPDELDELFLDSCALDCLEDVKKSVDVVLEKYRYDRKFPVGNGSEEKSLTDLRKVLGTEDVGCVYYRLIQAEIAHHMVEDFDESLLPGDAYEMICKGFFKDLELRSKYFYLDSLDSCPITCITQAVSTRTFNDQQFFQCFKSLLLQMNAGKLAGKYSHYKNKCLNFKIDRERLMNDVRISERESNSEALGKALSLTNCTTAVLKNLCFYSQESPQSYTSLGPDTGRLKFSLSYKEQVGGNRELYIGDLRTKMFTRLIEDYFEALTKQYRGSCLNNEKEFHNAILAMKLNVSLGQVSYSLDHSKWGPMMSPFLFLVFLQNLRWETGDDIEDIKSKDYVSTLLSWHIHKLIEVPFNVVNAMMRSYLKSRLGLKKSLHQTSTEAFFFEYFKQNRIPSHLSSIIDMGQGILHNASDFYGLVSERFINYCIKCLFEDEVDSYTSSDDQISLFGKDLSDLLSNEPEEFQAILEFHYFLSDQLNKFISPKSVIGSFVAEFKSRFYVWGDEVPLLTKFVAAALHNVKCKEPHQLAETIDTIIDQSVANGVPVTLCNAIQERTLNLLRYAQYPIDPFLLFLDSDVKDWVDGNRGYRIMRNIEAILPESTQKVRKVLRTVFNKLKLGELHEEFTAIYLSGDPADSFKKLTSLVGDDTLSEEDLSVCWLNLTTHHPLKMVMRQKVIYTGAVELGEEKLPTLVKTLQSKLSSNFTRGAQKLLCEAVNKSAFQSGIASGFIGLCKTLGSKCVRFSDRSTAYIKSLVSRLSALDSVSSLKVKGVDLWILGKEHTKAAEEALGFLRPVLWDYFCIALSTSLELGSWVLGEPKVKEKTSSIPFKPCDYFPMKPTTTKLLEDKVGFNHIIHSFRRLYPSLFERHLLPFMSDLASTKMRWTPRIKFLDLCVVLDVNCEAMSLISHVVKWKREEHYVVLSSDLAIAHERSHLPITDERVVTTYDVVQNFLRQIYFESFIRPFVATSRTLGSFTWFPHRSSIPESEGLDNLGPFSSFIEKVIYKGVERPMYRHDLYSGYAWLDFECAPAILNLGQLIASGLTEQHVFESVSELLEAFADLSVGSVQISVTVNFQVRSQGESLKEKFSLHLLFKGVVLEGGLFKPHSLDVTYSGSVQRSAIKDCWRVAQTSTWFKRETTSIWLLSTENICDYLRDSSPIPDVIPLSVLLNEEILDLEEHDFTHIGPEHVEIPLVVDSGYLIEGTRKLLPFNPNIHDQDLNVFIGELMEDHSEILERSLSKMLRSRMDQGLHWLQLDIIGVVGRCMPEGYENFLTRVFSGIDFWADFKGYSLCYSRSQASLMIQSSEGKFRLRGRLCRPLFEEVGPPLDIE

SEQ ID NO: 7 - protein, 15 aa, Mopeia mammarenavirus
PNAKTWIDIEGRPED

SEQ ID NO: 8 - protein, 7 aa, Mopeia mammarenavirus
DEGHDHD

SEQ ID NO: 9 - protein, 7 aa, Mopeia mammarenavirus
AEAHDHD

SEQ ID NO: 10 - protein, 7 aa, Mopeia mammarenavirus
AAAHDHD

SEQ ID NO: 11 - protein, 7 aa, Mopeia mammarenavirus
AAAADHD

SEQ ID NO: 12 - protein, 7 aa, Mopeia mammarenavirus
AAAAAHD

SEQ ID NO: 13 - protein, 7 aa, Mopeia mammarenavirus
AAAAAAD

SEQ ID NO: 14 - protein, 7 aa, Mopeia mammarenavirus
AAAAAHA

SEQ ID NO: 15 - protein, 7 aa, Mopeia mammarenavirus
AAAAAAA

SEQ ID NO: 16 - protein, 491 aa, Lassa mammarenavirus
MGQIVTFFQEVPHVIEEVMNIVLIALSVLAVLKGLYNFATCGLVGLVTFLLLCGRSCTTSLYKGVYELQTLELNMETLNMTMPLSCTKNNSHHYIMVGNETGLELTLTNTSIINHKFCNLSDAHKKNLYDHALMSIISTFHLSIPNFNQYEAMSCDFNGGKISVQYNLSHSYAGDAANHCGTVANGVLQTFMRMAWGGSYIALDSGRGNWDCIMTSYQYLIIQNTTWEDHCQFSRPSPIGYLGLLSQRTRDIYISRRLLGTFTWTLSDSEGKDTPGGYCLTRWMLIEAELKCFGNTAVAKCNEKHDEEFCDMLRLFDFNKQAIQRLKAEAQMSIQLINKAVNALINDQLIMKNHLRDIMGIPYCNYSKYWYLNHTTTGRTSLPKCWLVSNGSYLNETHFSDDIEQQADNMITEMLQKEYMERQGKTPLGLVDLFVFSTSFYLISIFLHLVKIPTHRHIVGKSCPKPHRLNHMGICSCGLYKQPGVPVKWKR

SEQ ID NO: 17 - protein, 454 aa, Lujo mammarenavirus
MGQIVAVFQAIPEILNEAINIVIIVIIMFTLIKGVFNLYKSGLFQLVIFLLLCGKRCDSSLLSGFNLETVHFNMSLLSSIPMVSEQQHCIQHNHSSITFSLLTNKSDLEKCNFTRLQAVDRVIFDLFREFHHRVGDFPVTSDLKCSHNTSYRVIEYEVTKESLPRLQEAVSTLFPDLHLSEDRFLQIQAHDDKNCTGLHPLNYLRLLKENSETHYKVRKLMKLFQWSLSDETGSPLPGGHCLERWLIFASDIKCFDNAAIAKCNKEHDEEFCDMLRLFDYNKASIAKLRGEASSSINLLSGRINAIISDTLLMRSSLKRLMGIPYCNYTKFWYLNHTKLGIHSLPRCWLVSNGSYLNETKFTHDMEDEADKLLTEMLKKEYVRRQEKTPITLMDILMFSVSFYMFSVTLCICNIPTHRHITGLPCPKPHRLRKNGTCACGFFKSINRSTGWAKH

SEQ ID NO: 18 - protein, 496 aa, Machupo mammarenavirus
MGQLISFFQEIPVFLQEALNIALVAVSLIAVIKGIINLYKSGLFQFIFFLLLAGRSCSDGTFKIGLHTEFQSVTLTMQRLLANHSNELPSLCMLNNSFYYMRGGVNTFLIRVSDISVLMKEYDVSIYEPEDLGNCLNKSDSSWAIHWFSNALGHDWLMDPPMLCRNKTKKEGSNIQFNISKADDARVYGKKIRNGMRHLFRGFHDPCEEGKVCYLTINQCGDPSSFDYCGVNHLSKCQFDHVNTLHFLVRSKTHLNFERSLKAFFSWSLTDSSGKDMPGGYCLEEWMLIAAKMKCFGNTAVAKCNQNHDSEFCDMLRLFDYNKNAIKTLNDESKKEINLLSQTVNALISDNLLMKNKIKELMSIPYCNYTKFWYVNHTLTGQHTLPRCWLIRNGSYLNTSEFRNDWILESDHLISEMLSKEYAERQGKTPITLVDICFWSTIFFTASLFLHLVGIPTHRHLKGEACPLPHKLDSFGGCRCGKYPRLKKPTIWHKRH

SEQ ID NO: 19 - protein, 479 aa, Guanarito mammarenavirus
MGQLISFFQDIPIFFEEALNVALAVVTLLAIIKGIVNVWKSGILQLFVFLVLAGRSCSFKVGHHTNFESFTVKLGGVFHELPSLCRVNNSYSLIRLSHNSNQALSVEYVDVHPVLCSSSPTILDNYTQCIKGSPEFDWILGWTIKGLGHDFLRDPRICCEPKKTTNAEFTFQLNLTDSPETHHYRSKIEVGIRHLFGNYITNDSYSKMSVVMRNTTWEGQCSNSHVNTLRFLVKNAGYLVGRKPLAFFSWSLSDPKGNDMPGGYCLERWMLVAGDLKCFGNTAVAKCNLNHDSEFCDMLRLFDFNKNAIEKLNNQTKTAVNMLTHSINSLISDNLLMRNKLKEILKVPYCNYTRFWYINHTKSGEHSLPRCWLVSNGSYLNESDFRNEWILESDHLIAEMLSKEYQDRQGKTPLTLVDLCFWSAIFFTTSLFLHLVGFPTHRHIQGDPCPLPHRLDRNGACRCGRFQKLGKQVTWKRKH

SEQ ID NO: 20 - protein, 484 aa, Chapare mammarenavirus
MGQLVSFFQEIPNIIQEAINIALIAVSLIAILKGLVNLWKSGLFQLLVFLILAGRSCSFKIGRSTELQNITINMLKVFEDHPISCTVNKTLYYIRESENATWCVEIAALDMSVLLSPHDPRVMGNLSNCVHPDIKHRSELLGLLEWILRALKYDFLNYPPLLCEKVTSSVNETRIQINVSDSAGSHDFKETMLQRLAILFGTKLMFDKTPKQFIVIRNQTWVNQCKSNHVNTLHLMMANAGHAVKLRRLQGVFTWTITDAAGNDMPGGYCLERWMLVTSDLKCFGNTALAKCNLNHDSEFCDMLKLFEFNKKAIESLNDNTKNKVNLLTHSINALISDNLLMKNRLKELLDTPYCNYTKFWYVNHTITGEHSLPRCWMVKNNSYLNESEFRNDWILESDHLLSEMLNKEYFDRQGKTPITLVDICFWSTLFFTTTLFLHLVGFPTHRHIQGEPCPLPHKLNSNGGCRCGRYPELKKPTTWHRKH

SEQ ID NO: 21 - protein, 488 aa, Sabia mammarenavirus
MGQLFSFFEEVPNIIHEAINIALIAVSLIAALKGMINLWKSGLFQLIFFLTLAGRSCSFRIGRSTELQNITFDMLKVFEDHPTSCMVNHSTYYVHENKNATWCLEVSVTDVTLLMAEHDRQVLNNLSNCVHPAVEHRSRMVGLLEWIFRALKYDFNHDPTPLCQKQTSTVNETRVQINITEGFGSHGFEDTILQRLGVLFGSRIAFSNIQDLGKKRFLLIRNSTWKNQCEMNHVNSMHLMLANAGRSSGSRRPLGIFSWTITDAVGNDMPGGYCLERWMLVTSDLKCFGNTALAKCNLDHDSEFCDMLKLFEFNKKAIETLNDNTKNKVNLLTHSINALISDNLLMKNRLKELLNTPYCNYTKFWYVNHTASGEHSLPRCWLVRNNSYLNESEFRNDWIIESDHLLSEMLNKEYIDRQGKTPLTLVDICFWSTLFFTTTLFLHLVGFPTHRHIRGEPCPLPHRLNSRGGCRCGKYPELKKPITWHKNH